European Patent Application EP 4 218 833 A1, published August 2, 2023. Title: LABELING OF ANTIBODIES. Applicant: WHITEHEAD INSTITUTE FOR BIOMEDICAL RESEARCH; THE GENERAL HOSPITAL CORPORATION D/B/A MASSACHUSETTS GENERAL HOSPITAL. The sequence listing filed with the application follows.

SEQUENCE LISTING (99 sequences)

SEQ ID NO: 1 - DNA, 378 bp, synthetic construct
  misc_feature 1..378: note = Synthetic Polynucleotide
  source 1..378: mol_type = other DNA
caggtgcagctgcaggagtcagggggaggattggtgcagcctggggggtctctgagactctcctgtacagcctctggattcacattcagtacttactacatgagctgggtccgcaaggctccagggaaggggcccgagtgggtctcagttatgaatagtagtggtggtgacacaaggtatgcagacttcgtgaagggccgattcaccatctccagagacaacgccaagaacacactgtatctccaaatgaacagcctgaaacctgaggatacggccctgtattactgtgcgcaaggtagatcagatatatacccaaccttcacgcggggccaggggacccaggtcaccgtctcctcaggaggactgccggaaaccggc

SEQ ID NO: 2 - protein, 133 aa, synthetic construct
  REGION 1..133: note = Synthetic Polypeptide
QVQLQESGGGLVQPGGSLRLSCTASGFTFSTYYMSWVRKAPGKGPEWVSVMNSSGGDTRYADFVKGRFTISRDNAKNTLYLQMNSLKPEDTALYYCAQGRSDIYPTFTRGQGTQVTVSSGSLPETGGHHHHHH

SEQ ID NO: 3 - DNA, 411 bp, synthetic construct
  misc_feature 1..411: note = Synthetic Polynucleotide
  source 1..411: mol_type = other DNA
caggttcaactgcaagagagtggcgggggcctggttcagaccggtggttctctccggctctcgtgtgccgcaagtggagtagattttaactggtatagcatgggttggttcaggcaagcccctggcaaagagcgggagtatgtggcttcgattgaccagggaggcgagttggattacgcaatatcagtaaagggcagattcacgatctcccgagacaacgcgaagaatatggtgtatctccagatgaattcgttaaagcccgaagacaccgctgtatactactgtgccgcagatttttccggccggggtgcgtcaaaccctgacaagtataaatattggggacagggaacccaagtgaccgtcagcagcggtgggttgcccgaaactggaggacaccatcaccatcaccat

SEQ ID NO: 4 - protein, 137 aa, synthetic construct
  REGION 1..137: note = Synthetic Polypeptide
QVQLQESGGGLVQTGGSLRLSCAASGVDFNWYSMGWFRQAPGKEREYVASIDQGGELDYAISVKGRFTISRDNAKNMVYLQMNSLKPEDTAVYYCAADFSGRGASNPDKYKYWGQGTQVTVSSGGLPETGGHHHHHH

SEQ ID NO: 5 - protein, 12 aa, synthetic construct
  REGION 1..12: note = Synthetic Polypeptide
LPETGGHHHHHH

SEQ ID NO: 6 - protein, 8 aa, synthetic construct
  REGION 1..8: note = Synthetic Polypeptide
GGHHHHHH

SEQ ID NO: 7 - protein, 4 aa, synthetic construct
  REGION 1..4: note = Synthetic Polypeptide
LPET

SEQ ID NO: 8 - protein, 7 aa, synthetic construct
  REGION 1..7: note = Synthetic Polypeptide
LPETGGG

SEQ ID NO: 9 - protein, 7 aa, synthetic construct
  REGION 1..7: note = Synthetic Polypeptide
  REGION 6..7: note = misc_feature - X can be any naturally occurring amino acid
LPETGXX

SEQ ID NO: 10 - protein, 8 aa, synthetic construct
  REGION 1..8: note = Synthetic Polypeptide
LPETGGGC

SEQ ID NO: 11 - protein, 5 aa, synthetic construct
  REGION 1..5: note = Synthetic Polypeptide
LPETG

SEQ ID NO: 12 - protein, 4 aa, synthetic construct
  REGION 1..4: note = Synthetic Polypeptide
GGGC

SEQ ID NO: 13 - protein, 6 aa, synthetic construct
  REGION 1..6: note = Synthetic Polypeptide
  SITE 3: note = misc_feature - X can be any naturally occurring amino acid
  SITE 6: note = misc_feature - X can be any naturally occurring amino acid
LPXTGX

SEQ ID NO: 14 - protein, 7 aa, synthetic construct
  REGION 1..7: note = Synthetic Polypeptide
  SITE 3: note = misc_feature - X can be any naturally occurring amino acid
LPXTGGG

SEQ ID NO: 15-16 - skipped (2 entries)

SEQ ID NO: 17 - protein, 5 aa, synthetic construct
  REGION 1..5: note = Synthetic Polypeptide
  SITE 3: note = misc_feature - X can be any naturally occurring amino acid
LPXAG

SEQ ID NO: 18 - protein, 5 aa, synthetic construct
  REGION 1..5: note = Synthetic Polypeptide
LPETA

SEQ ID NO: 19 - protein, 5 aa, synthetic construct
  REGION 1..5: note = Synthetic Polypeptide
NPQTN

SEQ ID NO: 20 - protein, 5 aa, synthetic construct
  REGION 1..5: note = Synthetic Polypeptide
NPKTG

SEQ ID NO: 21 - protein, 5 aa, synthetic construct
  REGION 1..5: note = Synthetic Polypeptide
LPSTG

SEQ ID NO: 22 - skipped

SEQ ID NO: 23 - protein, 5 aa, synthetic construct
  REGION 1..5: note = Synthetic Polypeptide
LPKTG

SEQ ID NO: 24 - protein, 5 aa, synthetic construct
  REGION 1..5: note = Synthetic Polypeptide
LPATG

SEQ ID NO: 25 - protein, 5 aa, synthetic construct
  REGION 1..5: note = Synthetic Polypeptide
LPNTG

SEQ ID NO: 26 - protein, 5 aa, synthetic construct
  REGION 1..5: note = Synthetic Polypeptide
LPNAG

SEQ ID NO: 27 - protein, 5 aa, synthetic construct
  REGION 1..5: note = Synthetic Polypeptide
  SITE 3: note = misc_feature - X can be any naturally occurring amino acid
LPXTA

SEQ ID NO: 28 - protein, 5 aa, synthetic construct
  REGION 1..5: note = Synthetic Polypeptide
LPNTA

SEQ ID NO: 29 - protein, 5 aa, synthetic construct
  REGION 1..5: note = Synthetic Polypeptide
LPETA

SEQ ID NO: 30 - protein, 5 aa, synthetic construct
  REGION 1..5: note = Synthetic Polypeptide
  SITE 3: note = misc_feature - X can be any naturally occurring amino acid
LGXTG

SEQ ID NO: 31 - protein, 5 aa, synthetic construct
  REGION 1..5: note = Synthetic Polypeptide
LGATG

SEQ ID NO: 32 - protein, 5 aa, synthetic construct
  REGION 1..5: note = Synthetic Polypeptide
  SITE 3: note = misc_feature - X can be any naturally occurring amino acid
IPXTG

SEQ ID NO: 33 - protein, 5 aa, synthetic construct
  REGION 1..5: note = Synthetic Polypeptide
IPNTG

SEQ ID NO: 34 - protein, 5 aa, synthetic construct
  REGION 1..5: note = Synthetic Polypeptide
IPETG

SEQ ID NO: 35 - skipped

SEQ ID NO: 36 - protein, 5 aa, synthetic construct
  REGION 1..5: note = Synthetic Polypeptide
NPQTN

SEQ ID NO: 37 - protein, 5 aa, synthetic construct
  REGION 1..5: note = Synthetic Polypeptide
NPKTG

SEQ ID NO: 38 - protein, 5 aa, synthetic construct
  REGION 1..5: note = Synthetic Polypeptide
NSKTA

SEQ ID NO: 39 - protein, 5 aa, synthetic construct
  REGION 1..5: note = Synthetic Polypeptide
NPQTG

SEQ ID NO: 40 - protein, 5 aa, synthetic construct
  REGION 1..5: note = Synthetic Polypeptide
NAKTN

SEQ ID NO: 41 - protein, 5 aa, synthetic construct
  REGION 1..5: note = Synthetic Polypeptide
NPQSS

SEQ ID NO: 42 - protein, 5 aa, synthetic construct
  REGION 1..5: note = Synthetic Polypeptide
  SITE 3: note = misc_feature - X is Glu, Ala, Ser, or His
NAXTG

SEQ ID NO: 43 - protein, 5 aa, synthetic construct
  REGION 1..5: note = Synthetic Polypeptide
  SITE 3: note = misc_feature - X can be any naturally occurring amino acid
LPXTA

SEQ ID NO: 44 - protein, 5 aa, synthetic construct
  REGION 1..5: note = Synthetic Polypeptide
  SITE 3: note = misc_feature - X can be any naturally occurring amino acid
LAXTG

SEQ ID NO: 45 - protein, 6 aa, synthetic construct
  REGION 1..6: note = Synthetic Polypeptide
QVPTGV

SEQ ID NO: 46 - protein, 5 aa, synthetic construct
  REGION 1..5: note = Synthetic Polypeptide
  SITE 3: note = misc_feature - X can be any naturally occurring amino acid
TLXTC

SEQ ID NO: 47 - protein, 206 aa, Staphylococcus aureus
MKKWTNRLMTIAGVVLILVAAYLFAKPHIDNYLHDKDKDEKIEQYDKNVKEQASKDNKQQAKPQIPKDKSKVAGYIEIPDADIKEPVYPGPATPEQLNRGVSFAEENESLDDQNISIAGHTFIDRPNYQFTNLKAAKKGSMVYFKVGNETRKYKMTSIRDVKPTDVEVLDEQKGKDKQLTLITCDDYNEKTGVWEKRKIFVATEVK

SEQ ID NO: 48 - protein, 206 aa, Staphylococcus aureus
MKKWTNRLMTIAGVVLILVAAYLFAKPHIDNYLHDKDKDEKIEQYDKNVKEQASKDKKQQAKPQIPKDKSKVAGYIEIPDADIKEPVYPGPATPEQLNRGVSFAEENESLDDQNISIAGHTFIDRPNYQFTNLKAAKKGSMVYFKVGNETRKYKMTSIRDVKPTDVGVLDEQKGKDKQLTLITCDDYNEKTGVWEKRKIFVATEVK

SEQ ID NO: 49 - protein, 148 aa, synthetic construct
  REGION 1..148: note = Synthetic Polypeptide
MQAKPQIPKDKSKVAGYIEIPDADIKEPVYPGPATREQLNRGVSFAEENESLDDQNISIAGHTFIDRPNYQFTNLKAAKKGSMVYFKVGNETRKYKMTSIRNVKPTAVEVLDEQKGKDKQLTLITCDDYNEETGVWETRKIFVATEVK

SEQ ID NO: 50 - protein, 6 aa, synthetic construct
  REGION 1..6: note = Synthetic Polypeptide
  SITE 3: note = misc_feature - X is Gln or Lys
  SITE 5: note = misc_feature - X is Ala or Ser
LPXTXT

SEQ ID NO: 51 - skipped

SEQ ID NO: 52 - protein, 5 aa, synthetic construct
  REGION 1..5: note = Synthetic Polypeptide
LPSTS

SEQ ID NO: 53 - protein, 5 aa, synthetic construct
  REGION 1..5: note = Synthetic Polypeptide
LPITG

SEQ ID NO: 54 - protein, 5 aa, synthetic construct
  REGION 1..5: note = Synthetic Polypeptide
LPDTA

SEQ ID NO: 55 - protein, 5 aa, synthetic construct
  REGION 1..5: note = Synthetic Polypeptide
SPKTG

SEQ ID NO: 56 - protein, 5 aa, synthetic construct
  REGION 1..5: note = Synthetic Polypeptide
LAETG

SEQ ID NO: 57 - protein, 5 aa, synthetic construct
  REGION 1..5: note = Synthetic Polypeptide
LAATG

SEQ ID NO: 58 - protein, 5 aa, synthetic construct
  REGION 1..5: note = Synthetic Polypeptide
LAHTG

SEQ ID NO: 59 - protein, 5 aa, synthetic construct
  REGION 1..5: note = Synthetic Polypeptide
LASTG

SEQ ID NO: 60 - protein, 5 aa, synthetic construct
  REGION 1..5: note = Synthetic Polypeptide
LPLTG

SEQ ID NO: 61 - protein, 5 aa, synthetic construct
  REGION 1..5: note = Synthetic Polypeptide
LSRTG

SEQ ID NO: 62 - protein, 5 aa, synthetic construct
  REGION 1..5: note = Synthetic Polypeptide
VPDTG

SEQ ID NO: 63 - protein, 5 aa, synthetic construct
  REGION 1..5: note = Synthetic Polypeptide
IPQTG

SEQ ID NO: 64 - protein, 5 aa, synthetic construct
  REGION 1..5: note = Synthetic Polypeptide
YPRRG

SEQ ID NO: 65 - protein, 5 aa, synthetic construct
  REGION 1..5: note = Synthetic Polypeptide
LPMTG

SEQ ID NO: 66 - protein, 5 aa, synthetic construct
  REGION 1..5: note = Synthetic Polypeptide
LAFTG

SEQ ID NO: 67 - protein, 5 aa, synthetic construct
  REGION 1..5: note = Synthetic Polypeptide
LPQTS

SEQ ID NO: 68-72 - skipped (5 entries)

SEQ ID NO: 73 - protein, 4 aa, synthetic construct
  REGION 1..4: note = Synthetic Polypeptide
NPQS

SEQ ID NO: 74 - protein, 4 aa, synthetic construct
  REGION 1..4: note = Synthetic Polypeptide
LPST

SEQ ID NO: 75 - protein, 4 aa, synthetic construct
  REGION 1..4: note = Synthetic Polypeptide
NSKT

SEQ ID NO: 76 - protein, 4 aa, synthetic construct
  REGION 1..4: note = Synthetic Polypeptide
NPQT

SEQ ID NO: 77 - protein, 4 aa, synthetic construct
  REGION 1..4: note = Synthetic Polypeptide
NAKT

SEQ ID NO: 78 - protein, 4 aa, synthetic construct
  REGION 1..4: note = Synthetic Polypeptide
LPIT

SEQ ID NO: 79 - protein, 4 aa, synthetic construct
  REGION 1..4: note = Synthetic Polypeptide
LAET

SEQ ID NO: 80 - protein, 4 aa, synthetic construct
  REGION 1..4: note = Synthetic Polypeptide
NPQS

SEQ ID NO: 81 - protein, 5 aa, synthetic construct
  REGION 1..5: note = Synthetic Polypeptide
  SITE 3: note = misc_feature - X can be any naturally occurring amino acid
LPXTG

SEQ ID NO: 82 - protein, 8 aa, synthetic construct
  REGION 1..8: note = Synthetic polypeptide
  VARIANT 3: note = X can be any naturally occurring amino acid
LPXTGGGK

SEQ ID NO: 83 - protein, 7 aa, synthetic construct
  REGION 1..7: note = Synthetic polypeptide
  VARIANT 3: note = X can be any naturally occurring amino acid
LPXTGGG

SEQ ID NO: 84 - protein, 8 aa, synthetic construct
  REGION 1..8: note = Synthetic polypeptide
  VARIANT 3: note = X can be any naturally occurring amino acid
NPXTGGGK

SEQ ID NO: 85 - protein, 7 aa, synthetic construct
  REGION 1..7: note = Synthetic polypeptide
  VARIANT 3: note = X can be any naturally occurring amino acid
NPXTGGG

SEQ ID NO: 86 - protein, 7 aa, synthetic construct
  REGION 1..7: note = Synthetic polypeptide
  VARIANT 3: note = X can be any naturally occurring amino acid
LPXTAAA

SEQ ID NO: 87 - protein, 7 aa, synthetic construct
  REGION 1..7: note = Synthetic polypeptide
  VARIANT 3: note = X can be any naturally occurring amino acid
NPXTAAA

SEQ ID NO: 88 - protein, 9 aa, synthetic construct
  REGION 1..9: note = Synthetic polypeptide
  VARIANT 3: note = X can be any naturally occurring amino acid
LPXTGGGGG

SEQ ID NO: 89 - protein, 5 aa, synthetic construct
  REGION 1..5: note = Synthetic polypeptide
LPGAG

SEQ ID NO: 90 - protein, 11 aa, synthetic construct
  REGION 1..11: note = Synthetic polypeptide
DSLEFIASKLA

SEQ ID NO: 91 - protein, 13 aa, synthetic construct
  REGION 1..13: note = Synthetic polypeptide
VLDSLEFIASKLA

SEQ ID NO: 92 - protein, 17 aa, synthetic construct
  REGION 1..17: note = Synthetic polypeptide
GSQDVLDSLEFIASKLA

SEQ ID NO: 93 - protein, 8 aa, synthetic construct
  REGION 1..8: note = Synthetic polypeptide
GGGSLLQG

SEQ ID NO: 94 - protein, 7 aa, synthetic construct
  REGION 1..7: note = Synthetic polypeptide
PNPQLPF

SEQ ID NO: 95 - protein, 7 aa, synthetic construct
  REGION 1..7: note = Synthetic polypeptide
PKPQQFM

SEQ ID NO: 96 - protein, 6 aa, synthetic construct
  REGION 1..6: note = Synthetic polypeptide
GQQQLG

SEQ ID NO: 97 - protein, 6 aa, synthetic construct
  REGION 1..6: note = Synthetic polypeptide
MRHKGS

SEQ ID NO: 98 - protein, 15 aa, synthetic construct
  REGION 1..15: note = Synthetic polypeptide
GLNDIFEAQKIEWHE

SEQ ID NO: 99 - protein, 13 aa, synthetic construct
  REGION 1..13: note = Synthetic polypeptide
GFEIDKVWYDLDA